European Patent Application EP 4 234 573 A1, published August 30, 2023. Title: Fusion Protein Comprising BP26 and Antigen Polypeptide. Applicant: Korea Advanced Institute of Science and Technology. The sequence listing filed with the application follows.

SEQUENCE LISTING (15 sequences)

SEQ ID NO: 1 - protein, 222 aa, Artificial Sequence
  BP26
QENQMTTQPARIAVTGEGMMTASPDMAILNLSVLRQAKTAREAMTANNEAMTKVLDAMKKAGIEDRDLQTGGIDIQPIYVYPDDKNNLKEPTITGYSVSTSLTVRVRELANVGKILDESVTLGVNQGGDLNLVNDNPSAVINEARKRAVANAIAKAKTLADAAGVGLGRVVEISELSRPPMPMPIARGQFRTMLAAAPDNSVPIAAGENSYNVSVNVVFEIK

SEQ ID NO: 2 - protein, 264 aa, Artificial Sequence
  BP26 comprising His tag and TEV cleavage site
MGSSHHHHHHSSGLVPRGSHMASMTGGQQMGRGSENLYFQGSQENQMTTQPARIAVTGEGMMTASPDMAILNLSVLRQAKTAREAMTANNEAMTKVLDAMKKAGIEDRDLQTGGIDIQPIYVYPDDKNNLKEPTITGYSVSTSLTVRVRELANVGKILDESVTLGVNQGGDLNLVNDNPSAVINEARKRAVANAIAKAKTLADAAGVGLGRVVEISELSRPPMPMPIARGQFRTMLAAAPDNSVPIAAGENSYNVSVNVVFEIK

SEQ ID NO: 3 - protein, 23 aa, Artificial Sequence
  M2e
SLLTEVETPIRNEWGSRSNDSSD

SEQ ID NO: 4 - protein, 23 aa, Artificial Sequence
  M2e(A/PR/8)
SLLTEVETPIRNEWGCRCNDGSD

SEQ ID NO: 5 - protein, 23 aa, Artificial Sequence
  M2e(A/CA/04/09)
SLLTEVETPTRNGWECKCSDSSD

SEQ ID NO: 6 - protein, 23 aa, Artificial Sequence
  M2e(A/Aquatic bird/Korea)
SLLTEVETPTRSEWECRCSDSSD

SEQ ID NO: 7 - DNA, 69 bp, Artificial Sequence
  M2e
agcctgctgaccgaagtcgagactccgatccgtaatgaatggggctctcgttctaacgactcgtcggat

SEQ ID NO: 8 - protein, 27 aa, Artificial Sequence
  Amino acid sequence of M30
PSKPSFQEFVDWENVSPELNSTDQPFL

SEQ ID NO: 9 - DNA, 81 bp, Artificial Sequence
  Nucleotide sequence of M30 (1)
ccgagcaaaccgagcttccaagagtttgtggactgggaaaacgttagcccggagctgaacagcaccgatcaaccgttcctg

SEQ ID NO: 10 - DNA, 81 bp, Artificial Sequence
  Nucleotide sequence of M30 (2)
ccgagcaagccgagcttccaagaatttgtggactgggagaacgttagcccggaactgaacagcaccgaccaaccgtttctg

SEQ ID NO: 11 - DNA, 81 bp, Artificial Sequence
  Nucleotide sequence of M30 (3)
ccttctaagccgagcttccaggagtttgtggactgggagaatgtctctcctgagctgaacagcactgaccaaccgttcctg

SEQ ID NO: 12 - DNA, 81 bp, Artificial Sequence
  Nucleotide sequence of M30 (4)
ccttctaaaccgagcttccaggaatttgtggactgggaaaatgtgtctcctgaactgaacagcactgatcaaccgtttctg

SEQ ID NO: 13 - DNA, 81 bp, Artificial Sequence
  Nucleotide sequence of M30 (5)
ccttccaaaccgagcttccaggagtttgtggactgggaaaacgtatctcccgagctgaacagcacagaccaaccgttcctg

SEQ ID NO: 14 - DNA, 81 bp, Artificial Sequence
  Nucleotide sequence of M30 (6)
ccttcaaagccgagcttccaagagtttgtggactgggagaatgtgagcccggagctgaatagcaccgaccaaccgttcctg

SEQ ID NO: 15 - DNA, 20 bp, Artificial Sequence
  CpG oligodeoxynucleotide
tccatgacgttcctgacgtt